European Patent Application EP 4 458 983 A1, published November 6, 2024. Title: SINGLE MOLECULE NANOPORE SEQUENCING METHOD. Applicant: BGI SHENZHEN. Application CN. The sequence listing filed with the application follows.

SEQUENCE LISTING (17 sequences)

SEQ ID NO: 1 - protein, 16 aa, synthetic construct
  source 1..16: note = Amino acid sequence of Spytag003
RGVPHIVMVDAYKRYK

SEQ ID NO: 2 - protein, 439 aa, synthetic construct
  source 1..439: note = Wild-type amino acid sequence of DDA helicase
MTFDDLTEGQKNAFNIVMKAIKEKKHHVTINGPAGTGKTTLTKFIIEALISTGETGIILAAPTHAAKKILSKLSGKEASTIHSILKINPVTYECNVLFEQKEVPDLAKARVLICDEVSMYDRKLFKILLSTIPPWATIIGIGDNKQIRPVDPGENTAYISPFFTHKDFYQCELTEVKRSNAPIIDVATDVRNGKWIYDKVVDGHGVRGFTGDTALRDFMVNYFSIVKSLDDLFENRVMAFTNKSVDKLNSIIRKKIFETDKDFIVGEIIVMQEPLFKTYKIDGKPVSEIIFNNGQLVRIIEAEYTSTFVKARGVPGEYLIRHWDLTVETYGDDEYYREKIKIISSDEELYKFNLFLGKTCETYKNWNKGGKAPWSDFWDAKSQFSKVKALPASTFHKAQGMSVDRAFIYTPCIHYADVELAQQLLYVGVTRGRYDVFYV

SEQ ID NO: 3 - protein, 184 aa, synthetic construct
  source 1..184: note = Wild-type amino acid sequence of MspA
GLDNELSLVDGQDRTLTVQQWDTFLNGVFPLDRNRLTREWFHSGRAKYIVAGPGADEFEGTLELGYQIGFPWSLGVGINFSYTTPNILINNGNITAPPFGLNSVITPNLFPGVSISARLGNGPGIQEVATFSVRVSGAKGGVAVSNAHGTVTGAAGGVLLRPFARLIASTGDSVTTYGEPWNMN

SEQ ID NO: 4 - protein, 114 aa, synthetic construct
  source 1..114: note = Spycatcher003; note = Amino acid sequence of Spycatcher003
MVTTLSGLSGEQGPSGDMTTEEDSATHIKFSKRDEDGRELAGATMELRDSSGKTISTWISDGHVKDFYLYPGKYTFVETAAPDGYEVATPIEFTVNEDGQVTVDGEATEGDAHT

SEQ ID NO: 5 - protein, 6 aa, synthetic construct
  source 1..6: note = Thrombin recognition sequence
LVPRGS

SEQ ID NO: 6 - protein, 8 aa, synthetic construct
  source 1..8: note = Amino acid sequence of Strep tag
WSHPQFEK

SEQ ID NO: 7 - protein, 473 aa, synthetic construct
  source 1..473: note = Amino acid sequence of Spytag003-DDA
RGVPHIVMVDAYKRYKGGSGGSGGSGGSGGSGGSMTFDDLTEGQKNAFNIVMKAIKEKKHHVTINGPAGTGKTTLTKFIIEALISTGGTGIILAAPTHAAKKILSKLSGKEASTIHSILKINPVTYEENVLFEQKEVPDLAKCRVLICDEVSMYDRKLFKILLSTIPPWCTIIGIGDNKQIRPVEPGENTAYISPFFTHKDFYQCELTEVKRSNAPIIDVATDVRNGKWNYDKVVDGHGVRGFTGDTALRDFMVNYFSIVKSLDDLFENRVMAFTNKSVDKLNSIIRKKIFETDKDFIVGEIIVMQEPLFKTYKIDGKPVSEIIFNNGQLVRIIEAEYTSTFVKARGVPGEYLIRHWDLTVETYGDDEYYREKIKIISSDEELYKFNLFLAKTAETYKNWNKGGKAPWSDFWDAKSQFSKVKALPASTFHKAQGMSVDRAFIYTPCIHYADVELAQQLLYVGVTRGRYDVFYV

SEQ ID NO: 8 - protein, 307 aa, synthetic construct
  source 1..307: note = Amino acid sequence of Spycatcher003-MspA
MVTTLSGLSGEQGPSGDMTTEEDSATHIKFSKRDEDGRELAGATMELRDSSGKTISTWISDGHVKDFYLYPGKYTFVETAAPDGYEVATPIEFTVNEDGQVTVDGEATEGDAHTGGSGGSGGSGLDNELSLVDGQDRTLTVQQWDTFLNGVFPLDRNRLTREWFHSGRAKYIVAGPGADEFEGTLELGYQIGFPWSLGVGINFSYTTPNILIDDGDITAPPFGLNSVITPNLFPGVSISADLGNGPGIQEVATFSVDVSGAEGGVAVSNAHGTVTGAAGGVLLRPFARLIASTGDSVTTYGEPWNMN

SEQ ID NO: 9 - protein, 200 aa, synthetic construct
  source 1..200: note = Amino acid sequence of Strep-MspA
WSHPQFEKGALVPRGSGLDNELSLVDGQDRTLTVQQWDTFLNGVFPLDRNRLTREWFHSGRAKYIVAGPGADEFEGTLELGYQIGFPWSLGVGINFSYTTPNILIDDGDITAPPFGLNSVITPNLFPGVSISADLGNGPGIQEVATFSVDVSGAEGGVAVSNAHGTVTGAAGGVLLRPFARLIASTGDSVTTYGEPWNMN

SEQ ID NO: 10 - DNA, 68 bp, synthetic construct
  source 1..68: mol_type = other DNA; note = Top strand of adapter
ttttttttttttttttttttttttttttttttttttttttggttgtttctgttggtgctgatattgct

SEQ ID NO: 11 - DNA, 45 bp, synthetic construct
  source 1..45: mol_type = other DNA; note = Bottom strand of adapter
gcaatatcagcaccaacagaaacaacctttgaggcgagcggtcaa

SEQ ID NO: 12 - DNA, 15 bp, synthetic construct
  source 1..15: mol_type = other DNA; note = Sequence of tether
ttgaccgctcgcctc

SEQ ID NO: 13 - DNA, 2629 bp, synthetic construct
  source 1..2629: mol_type = other DNA; note = DNA sequence to be tested
ggcgtaatcatggtcatagctgtttcctgtgtgaaattgttatccgctcacaattccacacaacatacgagccggaagcataaagtgtaaagcctggggtgcctaatgagtgagctaactcacattaattgcgttgcgctcactgcccgctttccagtcgggaaacctgtcgtgccagctgcattaatgaatcggccaacgcgcggggagaggcggtttgcgtattgggcgctcttccgcttcctcgctcactgactcgctgcgctcggtcgttcggctgcggcgagcggtatcagctcactcaaaggcggtaatacggttatccacagaatcaggggataacgcaggaaagaacatgtgagcaaaaggccagcaaaaggccaggaaccgtaaaaaggccgcgttgctggcgtttttccataggctccgcccccctgacgagcatcacaaaaatcgacgctcaagtcagaggtggcgaaacccgacaggactataaagataccaggcgtttccccctggaagctccctcgtgcgctctcctgttccgaccctgccgcttaccggatacctgtccgcctttctcccttcgggaagcgtggcgctttctcatagctcacgctgtaggtatctcagttcggtgtaggtcgttcgctccaagctgggctgtgtgcacgaaccccccgttcagcccgaccgctgcgccttatccggtaactatcgtcttgagtccaacccggtaagacacgacttatcgccactggcagcagccactggtaacaggattagcagagcgaggtatgtaggcggtgctacagagttcttgaagtggtggcctaactacggctacactagaagaacagtatttggtatctgcgctctgctgaagccagttaccttcggaaaaagagttggtagctcttgatccggcaaacaaaccaccgctggtagcggtggtttttttgtttgcaagcagcagattacgcgcagaaaaaaaggatctcaagaagatcctttgatcttttctacggggtctgacgctcagtggaacgaaaactcacgttaagggattttggtcatgagattatcaaaaaggatcttcacctagatccttttaaattaaaaatgaagttttaaatcaatctaaagtatatatgagtaaacttggtctgacagttaccaatgcttaatcagtgaggcacctatctcagcgatctgtctatttcgttcatccatagttgcctgactccccgtcgtgtagataactacgatacgggagggcttaccatctggccccagtgctgcaatgataccgcgagacccacgctcaccggctccagatttatcagcaataaaccagccagccggaagggccgagcgcagaagtggtcctgcaactttatccgcctccatccagtctattaattgttgccgggaagctagagtaagtagttcgccagttaatagtttgcgcaacgttgttgccattgctacaggcatcgtggtgtcacgctcgtcgtttggtatggcttcattcagctccggttcccaacgatcaaggcgagttacatgatcccccatgttgtgcaaaaaagcggttagctccttcggtcctccgatcgttgtcagaagtaagttggccgcagtgttatcactcatggttatggcagcactgcataattctcttactgtcatgccatccgtaagatgcttttctgtgactggtgagtactcaaccaagtcattctgagaatagtgtatgcggcgaccgagttgctcttgcccggcgtcaatacgggataataccgcgccacatagcagaactttaaaagtgctcatcattggaaaacgttcttcggggcgaaaactctcaaggatcttaccgctgttgagatccagttcgatgtaacccactcgtgcacccaactgatcttcagcatcttttactttcaccagcgtttctgggtgagcaaaaacaggaaggcaaaatgccgcaaaaaagggaataagggcgacacggaaatgttgaatactcatactcttcctttttcaatattattgaagcatttatcagggttattgtctcatgagcggatacatatttgaatgtatttagaaaaataaacaaataggggttccgcgcacatttccccgaaaagtgccacctgacgtctaagaaaccattattatcatgacattaacctataaaaataggcgtatcacgaggccctttcgtctcgcgcgtttcggtgatgacggtgaaaacctctgacacatgcagctcccggagacggtcacagcttgtctgtaagcggatgccgggagcagacaagcccgtcagggcgcgtcagcgggtgttggcgggtgtcggggctggcttaactatgcggcatcagagcagattgtactgagagtgcaccatatgcggtgtgaaataccgcacagatgcgtaaggagaaaataccgcatcaggcgccattcgccattcaggctgcgcaactgttgggaagggcgatcggtgcgggcctcttcgctattacgccagctggcgaaagggggatgtgctgcaaggcgattaagttgggtaacgccagggttttcccagtcacgacgttgtaaaacgacggccagt

SEQ ID NO: 14 - protein, 18 aa, synthetic construct
  source 1..18: note = Amino acid sequence of Linker 1
GGSGGSGGSGGSGGSGGS

SEQ ID NO: 15 - protein, 9 aa, synthetic construct
  source 1..9: note = Amino acid sequence of Linker 2
GGSGGSGGS

SEQ ID NO: 16 - protein, 439 aa, synthetic construct
  source 1..439: note = Amino acid sequence of DDA helicase mutant
MTFDDLTEGQKNAFNIVMKAIKEKKHHVTINGPAGTGKTTLTKFIIEALISTGGTGIILAAPTHAAKKILSKLSGKEASTIHSILKINPVTYEENVLFEQKEVPDLAKCRVLICDEVSMYDRKLFKILLSTIPPWCTIIGIGDNKQIRPVEPGENTAYISPFFTHKDFYQCELTEVKRSNAPIIDVATDVRNGKWNYDKVVDGHGVRGFTGDTALRDFMVNYFSIVKSLDDLFENRVMAFTNKSVDKLNSIIRKKIFETDKDFIVGEIIVMQEPLFKTYKIDGKPVSEIIFNNGQLVRIIEAEYTSTFVKARGVPGEYLIRHWDLTVETYGDDEYYREKIKIISSDEELYKFNLFLAKTAETYKNWNKGGKAPWSDFWDAKSQFSKVKALPASTFHKAQGMSVDRAFIYTPCIHYADVELAQQLLYVGVTRGRYDVFYV

SEQ ID NO: 17 - protein, 184 aa, synthetic construct
  source 1..184: note = Amino acid sequence of MspA mutant
GLDNELSLVDGQDRTLTVQQWDTFLNGVFPLDRNRLTREWFHSGRAKYIVAGPGADEFEGTLELGYQIGFPWSLGVGINFSYTTPNILIDDGDITAPPFGLNSVITPNLFPGVSISADLGNGPGIQEVATFSVDVSGAEGGVAVSNAHGTVTGAAGGVLLRPFARLIASTGDSVTTYGEPWNMN